European Patent Specification EP 3 591 065 B1, published January 10, 2024. Title: Manufacture of recombinant Clostridium botulinum neurotoxins. Applicant: Ipsen Bionnovation Limited. The sequence listing filed with the application follows.

SEQUENCE LISTING (15 sequences)

SEQ ID NO: 1 - protein, 1296 aa, Clostridium Botulinum
MPFVNKQFNYKDPVNGVDIAYIKIPNAGQMQPVKAFKIHNKIWVIPERDTFTNPEEGDLNPPPEAKQVPVSYYDSTYLSTDNEKDNYLKGVTKLFERIYSTDLGRMLLTSIVRGIPFWGGSTIDTELKVIDTNCINVIQPDGSYRSEELNLVIIGPSADIIQFECKSFGHEVLNLTRNGYGSTQYIRFSPDFTFGFEESLEVDTNPLLGAGKFATDPAVTLAHELIHAGHRLYGIAINPNRVFKVNTNAYYEMSGLEVSFEELRTFGGHDAKFIDSLQENEFRLYYYNKFKDIASTLNKAKSIVGTTASLQYMKNVFKEKYLLSEDTSGKFSVDKLKFDKLYKMLTEIYTEDNFVKFFKVLNRKTYLNFDKAVFKINIVPKVNYTIYDGFNLRNTNLAANFNGQNTEINNMNFTKLKNFTGLFEFYKLLCVRGIITSKTKSLDKGYNKALNDLCIKVNNWDLFFSPSEDNFTNDLNKGEEITSDTNIEAAEENISLDLIQQYYLTFNFDNEPENISIENLSSDIIGQLELMPNIERFPNGKKYELDKYTMFHYLRAQEFEHGKSRIALTNSVNEALLNPSRVYTFFSSDYVKKVNKATEAAMFLGWVEQLVYDFTDETSEVSTTDKIADITIIIPYIGPALNIGNMLYKDDFVGALIFSGAVILLEFIPEIAIPVLGTFALVSYIANKVLTVQTIDNALSKRNEKWDEVYKYIVTNWLAKVNTQIDLIRKKMKEALENQAEATKAIINYQYNQYTEEEKNNINFNIDDLSSKLNESINKAMININKFLNQCSVSYLMNSMIPYGVKRLEDFDASLKDALLKYIYDNRGTLIGQVDRLKDKVNNTLSTDIPFQLSKYVDNQRLLSTFTEYIKNIINTSILNLRYESNHLIDLSRYASKINIGSKVNFDPIDKNQIQLFNLESSKIEVILKNAIVYNSMYENFSTSFWIRIPKYFNSISLNNEYTIINCMENNSGWKVSLNYGEIIWTLQDTQEIKQRVVFKYSQMINISDYINRWIFVTITNNRLNNSKIYINGRLIDQKPISNLGNIHASNNIMFKLDGCRDTHRYIWIKYFNLFDKELNEKEIKDLYDNQSNSGILKDFWGDYLQYDKPYYMLNLYDPNKYVDVNNVGIRGYMYLKGPRGSVMTTNIYLNSSLYRGTKFIIKKYASGNKDNIVRNNDRVYINVVVKNKEYRLATNASQAGVEKILSALEIPDVGNLSQVVVMKSKNDQGITNKCKMNLQDNNGNDIGFIGFHQFNNIAKLVASNWYNRQIERSSRTLGCSWEFIPVDDGWGERPL

SEQ ID NO: 2 - protein, 25 aa, Clostridium Botulinum
CVRGIITSKTKSLDKGYNKALNDLC

SEQ ID NO: 3 - protein, 25 aa, Clostridium Botulinum
CVRGIIPFKTKSLDEGYNKALNDLC

SEQ ID NO: 4 - protein, 25 aa, Clostridium Botulinum
CVRGIIPFKTKSLDEGYNKALNDLC

SEQ ID NO: 5 - protein, 25 aa, Clostridium Botulinum
CVRGIIPFKTKSLDEGYNKALNYLC

SEQ ID NO: 6 - protein, 25 aa, Clostridium Botulinum
CVRGIITSKTKSLDEGYNKALNELC

SEQ ID NO: 7 - protein, 25 aa, Clostridium Botulinum
CVRGIITSKTKSLDEGYNKALNDLC

SEQ ID NO: 8 - protein, 333 aa, Clostridium Botulinum
VQGQSVKGVGKTSLDGLVNIDVTYGNGKYYLKDSNKNIYLYDLKNQVDEYDLYNYLSRPNYKQILMSKSELISNYNNNFIANNQVNSVDAYVNTNKTYDYYKNKLNRNSIDNKGMNINGFVHVGRNYGNAFWYGPYDGMFFGDGDGIYFSSLAKSLDVVGHELSHGVTNKESNLKYENESGALNESFSDIMGVAVEGKNFVLGEDCWVAGGVMRDMENPSRGGQPAHMKDYKYKTMNDDNGGVHTNSGIINHAAYLVADGIEKTGAKNSKDIMGKIFYTANCYKWDETTNFAKCRNDVVQVTKELYGENSNYVKIVEKAFDQVGITATPQLPL

SEQ ID NO: 9 - protein, 581 aa, Clostridium Botulinum
MKSKKLLATVLSAVITFSTVSAVYAAPVGKESKVEPKTTTITWEKNEQNTKKAATDITEKKFNNSEEITKFFEKNISKFGVQKGSLKNTKTVKDEKGKTNYHMIYEVEGIPVYYGRIVFTTEKDSSMDSINGRIDTVFENGNWKNKIKLSKEDAIAKAKNDIKDEKATSKKTDLYLYNFEGKPYVVYLVDLITDNGSWTVFVNAEDGSIVNKFNNTPTLIDTKDQKLPNAKKIKDEAKKASNANNVIDVQGQSVKGVGKTSLDGLVNIDVTYGNGKYYLKDSNKNIYLYDLKNQVDEYDLYNYLSRPNYKQILMSKSELISNYNNNFIANNQVNSVDAYVNTNKTYDYYKNKLNRNSIDNKGMNINGFVHVGRNYGNAFWYGPYDGMFFGDGDGIYFSSLAKSLDVVGHELSHGVTNKESNLKYENESGALNESFSDIMGVAVEGKNFVLGEDCWVAGGVMRDMENPSRGGQPAHMKDYKYKTMNDDNGGVHTNSGIINHAAYLVADGIEKTGAKNSKDIMGKIFYTANCYKWDETTNFAKCRNDVVQVTKELYGENSNYVKIVEKAFDQVGITATPQLPL

SEQ ID NO: 10 - DNA, 1005 bp, Clostridium Botulinum
atggttcaaggtcaaagcgttaaaggagtaggaaaaactagcttggatggactagtaaatattgatgtaacttatggaaatggaaaatactatttaaaagatagcaacaaaaatatttatctatatgacttaaaaaatcaagttgatgaatatgatctatacaattatcttagtagacctaactataaacaaatattaatgagcaaatctgaattaatatctaattacaataataattttatagccaacaatcaggttaattctgtagatgcttatgtaaacacaaataaaacctatgattattataaaaacaaattaaatagaaacagtattgataataagggtatgaatattaatgggtttgttcatgtaggtagaaattatggtaatgctttttggtacggtccatatgatgggatgttctttggcgatggcgacggaatatacttctcttcccttgcaaaatctttagatgttgtaggccacgaattaagtcatggtgtaacaaataaagagtctaatcttaaatatgaaaatgaatctggtgccctaaatgaatctttctcagatattatgggagtagctgttgagggtaaaaactttgtactaggtgaagattgctgggttgctggaggagtaatgagagatatggaaaatccatccagaggaggccaaccagctcatatgaaagattataaatacaaaactatgaatgacgataacggtggtgttcatacaaattcaggtataataaaccatgctgcttatttagttgcagatggaatagaaaaaactggtgcaaaaaatagtaaagatattatgggaaaaatattctatacagctaattgctataaatgggatgaaacaacaaattttgctaagtgcagaaatgatgtagtccaagttactaaagaactttatggcgaaaatagcaactatgtaaaaattgttgaaaaagcttttgaccaagttggaataactgctacacctcaattaccattataa

SEQ ID NO: 11 - DNA, 1746 bp, Clostridium Botulinum
atgaaaagtaaaaaattattagctacagtgctaagtgccgtgatcactttttctactgtttctgcagtttatgctgcgcctgtaggaaaagaaagtaaagttgaaccaaaaactacaacaataacttgggaaaaaaatgaacaaaatactaaaaaagctgctactgatataactgaaaagaaatttaacaattctgaggagataactaaattctttgaaaaaaatatatctaaatttggtgtacaaaaaggttctcttaaaaacaccaagactgtaaaagacgaaaaaggtaaaactaactatcatatgatttatgaagtagaaggtatacctgtatactatggaagaattgtttttacaactgaaaaagactcctccatggattctataaacggtagaattgatactgtttttgaaaatgggaattggaaaaacaaaatcaaactatcaaaagaagatgctatagcaaaagctaaaaatgatattaaagatgaaaaagcaactagtaaaaagaccgatttatatctgtataattttgagggcaaaccttatgtagtttatttagtagatctaattacagacaacgggagttggacggttttcgttaatgctgaggatggttctatagtaaataaatttaataatactcctactttaattgatactaaagatcaaaaattacccaatgctaaaaaaattaaagatgaagctaaaaaagctagtaatgcaaataatgtaattgatgttcaaggtcaaagcgttaaaggagtaggaaaaactagcttggatggactagtaaatattgatgtaacttatggaaatggaaaatactatttaaaagatagcaacaaaaatatttatctatatgacttaaaaaatcaagttgatgaatatgatctatacaattatcttagtagacctaactataaacaaatattaatgagcaaatctgaattaatatctaattacaataataattttatagccaacaatcaggttaattctgtagatgcttatgtaaacacaaataaaacctatgattattataaaaacaaattaaatagaaacagtattgataataagggtatgaatattaatgggtttgttcatgtaggtagaaattatggtaatgctttttggtacggtccatatgatgggatgttctttggcgatggcgacggaatatacttctcttcccttgcaaaatctttagatgttgtaggccacgaattaagtcatggtgtaacaaataaagagtctaatcttaaatatgaaaatgaatctggtgccctaaatgaatctttctcagatattatgggagtagctgttgagggtaaaaactttgtactaggtgaagattgctgggttgctggaggagtaatgagagatatggaaaatccatccagaggaggccaaccagctcatatgaaagattataaatacaaaactatgaatgacgataacggtggtgttcatacaaattcaggtataataaaccatgctgcttatttagttgcagatggaatagaaaaaactggtgcaaaaaatagtaaagatattatgggaaaaatattctatacagctaattgctataaatgggatgaaacaacaaattttgctaagtgcagaaatgatgtagtccaagttactaaagaactttatggcgaaaatagcaactatgtaaaaattgttgaaaaagcttttgaccaagttggaataactgctacacctcaattaccattataa

SEQ ID NO: 12 - protein, 16 aa, Artificial Sequence
  Artificial Sequence
VPPTPGSAWSHPQFEK

SEQ ID NO: 13 - protein, 25 aa, Clostridium botulinum
CVRGIITSKTKSLDEGYNKALNDLC

SEQ ID NO: 14 - protein, 25 aa, Clostridium botulinum
CVRGIIPFKTKSLDEGYNKALNDLC

SEQ ID NO: 15 - protein, 1296 aa, Clostridium botulinum
MPFVNKQFNYKDPVNGVDIAYIKIPNAGQMQPVKAFKIHNKIWVIPERDTFTNPEEGDLNPPPEAKQVPVSYYDSTYLSTDNEKDNYLKGVTKLFERIYSTDLGRMLLTSIVRGIPFWGGSTIDTELKVIDTNCINVIQPDGSYRSEELNLVIIGPSADIIQFECKSFGHEVLNLTRNGYGSTQYIRFSPDFTFGFEESLEVDTNPLLGAGKFATDPAVTLAHELIHAGHRLYGIAINPNRVFKVNTNAYYEMSGLEVSFEELRTFGGHDAKFIDSLQENEFRLYYYNKFKDIASTLNKAKSIVGTTASLQYMKNVFKEKYLLSEDTSGKFSVDKLKFDKLYKMLTEIYTEDNFVKFFKVLNRKTYLNFDKAVFKINIVPKVNYTIYDGFNLRNTNLAANFNGQNTEINNMNFTKLKNFTGLFEFYKLLCVRGIITSKTKSLDKGYNKALNDLCIKVNNWDLFFSPSEDNFTNDLNKGEEITSDTNIEAAEENISLDLIQQYYLTFNFDNEPENISIENLSSDIIGQLELMPNIERFPNGKKYELDKYTMFHYLRAQEFEHGKSRIALTNSVNEALLNPSRVYTFFSSDYVKKVNKATEAAMFLGWVEQLVYDFTDETSEVSTTDKIADITIIIPYIGPALNIGNMLYKDDFVGALIFSGAVILLEFIPEIAIPVLGTFALVSYIANKVLTVQTIDNALSKRNEKWDEVYKYIVTNWLAKVNTQIDLIRKKMKEALENQAEATKAIINYQYNQYTEEEKNNINFNIDDLSSKLNESINKAMININKFLNQCSVSYLMNSMIPYGVKRLEDFDASLKDALLKYIYDNRGTLIGQVDRLKDKVNNTLSTDIPFQLSKYVDNQRLLSTFTEYIKNIINTSILNLRYESKHLIDLSRYASKINIGSKVNFDPIDKNQIQLFNLESSKIEVILKKAIVYNSMYENFSTSFWIRIPKYFNKISLNNEYTIINCMENNSGWKVSLNYGEIIWTLQDTKEIKQRVVFKYSQMINISDYINRWIFVTITNNRLNKSKIYINGRLIDQKPISNLGNIHASNKIMFKLDGCRDTHRYIWIKYFNLFDKELNEKEIKDLYDNQSNSGILKDFWGDYLQYDKPYYMLNLYDPNKYVDVNNVGIRGYMYLKGPRGSVMTTNIYLNSSLYRGTKFIIKKYASGNKDNIVRNNDRVYINVVVKNKEYRLATNASQAGVEKILSALEIPDVGNLSQVVVMKSKNDKGITNKCKMNLQDNNGNDIGFIGFHQFNNIAKLVASNWYNRQIERSSRTLGCSWEFIPVDDGWGERPL